European Patent Application EP 4 434 528 A1, published September 25, 2024. Title: THERAPEUTIC NUCLEIC ACID MOLECULE, MIXTURE, AND DRUG, AND USE THEREOF IN TREATING SOLID TUMOR. Applicant: LIVERNA THERAPEUTICS INC. Application WO. The sequence listing filed with the application follows.

SEQUENCE LISTING (52 sequences)

SEQ ID NO: 1 - RNA, 371 nt, synthetic construct
  source 1..371: mol_type = other RNA
gcgcctgcccacctgccaccgactgctggaacccagccagtgggagggcctggcccaccagagtcctgctccctcactcctcgccccgccccctgtcccagagtcccacctgggggctctctccacccttctcagagttccagtttcaaccagagttccaaccaatgggctccatcctctggattctggccaatgaaatatctccctggcagggtcctcttcttttcccagagctccaccccaaccaggagctctagttaatggagagctcccagcacactcggagcttgtgctttgtctccacgcaaagcgataaataaaagcattggtggcctttggtctttgaataaagcctgagtaggaagtctaga

SEQ ID NO: 2 - RNA, 568 nt, synthetic construct
  source 1..568: mol_type = other RNA
gcccctgccgctcccacccccacccatctgggccccgggttcaagagagagcggggtctgatctcgtgtagccatatagagtttgcttctgagtgtctgctttgtttagtagaggtgggcaggaggagctgaggggctggggctggggtgttgaagttggctttgcatgcccagcgatgcgcctccctgtgggatgtcatcaccctgggaaccgggagtggcccttggctcactgtgttctgcatggtttggatctgaattaattgtcctttcttctaaatcccaaccgaacttcttccaacctccaaactggctgtaaccccaaatccaagccattaactacacctgacagtagcaattgtctgattaatcactggccccttgaagacagcagaatgtccctttgcaatgaggaggagatctgggctgggcgggccagctggggaagcatttgactatctggaacttgtgtgtgcctcctcaggtatggcagtgactcacctggttttaataaaacaacctgcaacatctcatggtctttgaataaagcctgagtaggaagtctaga

SEQ ID NO: 3 - RNA, 289 nt, synthetic construct
  source 1..289: mol_type = other RNA
acacactccacctccagcacgcgacttctcaggacgacgaatcttctcaatgggggggcggctgagctccagccaccccgcagtcactttctttgtaacaacttccgttgctgccatcgtaaactgacacagtgtttataacgtgtacatacattaacttattacctcattttgttatttttcgaaacaaagccctgtggaagaaaatggaaaacttgaagaagcattaaagtcattctgttaagctgcgtaaatggtctttgaataaagcctgagtaggaagtctaga

SEQ ID NO: 4 - RNA, 379 nt, synthetic construct
  source 1..379: mol_type = other RNA
catcacatttaaaagcatctcagcctaccatgagaataagagaaagaaaatgaagatcaaaagcttattcatctgtttttctttttcgttggtgtaaagccaacaccctgtctaaaaaacataaatttctttaatcattttgcctcttttctctgtgcttcaattaataaaaaatggaaagaatctaatagagtggtacagcactgttatttttcaaagatgtgttgctatcctgaaaattctgtaggttctgtggaagttccagtgttctctcttattccacttcggtagaggatttctagtttcttgtgggctaattaaataaatcattaatactcttctaatggtctttgaataaagcctgagtaggaagtctaga

SEQ ID NO: 5 - RNA, 118 nt, synthetic construct
  source 1..118: mol_type = other RNA
gctgccttctgcggggcttgccttctggccatgcccttcttctctcccttgcacctgtacctcttggtctttgaataaagcctgagtaggaaggcggccgctcgagcatgcatctaga

SEQ ID NO: 6 - RNA, 297 nt, synthetic construct
  source 1..297: mol_type = other RNA
cgccgccgcccgggccccgcagtcgagggtcgtgagcccaccccgtccatggtgctaagcgggcccgggtcccacacggccagcaccgctgctcactcggacgacgccctgggcctgcacctctccagctcctcccacggggtccccgtagccccggcccccgcccagccccaggtctccccaggccctccgcaggctgcccggcctccctccccctgcagccatcccaaggctcctgacctacctggcccctgagctctggagcaagccctgacccaataaaggctttgaacccat

SEQ ID NO: 7 - RNA, 110 nt, synthetic construct
  source 1..110: mol_type = other RNA
gctggagcctcggtggccatgcttcttgccccttgggcctccccccagcccctcctccccttcctgcacccgtacccccgtggtctttgaataaagtctgagtgggcggc

SEQ ID NO: 8 - RNA, 116 nt, synthetic construct
  source 1..116: mol_type = other RNA
taataggctggagcctcggtggccatgcttcttgccccttgggcctccccccagcccctcctccccttcctgcacccgtacccccgtggtctttgaataaagtctgagtgggcggc

SEQ ID NO: 9 - RNA, 118 nt, synthetic construct
  source 1..118: mol_type = other RNA
tgataataggctggagcctcggtggccatgcttcttgccccttgggcctccccccagcccctcctccccttcctgcacccgtaccccctggtctttgaataaagtctgagtgggcggc

SEQ ID NO: 10 - RNA, 74 nt, synthetic construct
  source 1..74: mol_type = other RNA
ggactagttataagactgactagcccgatgggcctcccaacgggccctcctcccctccttgcaccgagattaat

SEQ ID NO: 11 - RNA, 1161 nt, synthetic construct
  source 1..1161: mol_type = other RNA
atgaaaatcctgaaaccttacatgagaaacacaagcatcagctgttacctgtgctttctgctgaacagccacttccttacagaggccggcatccacgtgttcatcctgggctgcgtgtccgtgggtctccctaagaccgaagctaattggatcgacgtgcggtacgacctggaaaagatcgagagcctgatccagagcatccacatcgacaccaccctgtatacagatagcgacttccaccccagctgcaaggtgaccgccatgaactgcttcctgctggaactgcaggtgatcctgcacgagtacagcaacatgacactgaatgagacagtgcggaacgtgctgtacctggccaactccacactgagctccaacaagaatgtggccgagagcggctgtaaagagtgcgaggaactggaggaaaagaccttcaccgagttcctgcagtcttttatccggatcgtgcagatgttcattaataccagctctggcggaggcagcggcggcggcggaagcggcggcggcggctctggaggcggaggaagcggcggcggcagcctgcaaggcaccacctgtcctccccccgtttctatcgagcacgccgacatcagagtgaagaactacagcgtcaacagccgggaaagatacgtgtgcaacagcggcttcaagagaaaggccggaaccagcacactgatcgaatgcgtgattaacaagaacaccaacgtggctcactggaccactcccagcctgaagtgcatcagagatcctagcctggcccactactccccagtgcccaccgtggtcacccctaaggtcacctcacagcctgagtcacccagccctagcgccaaggaacccgaggccttttctccaaaatctgatacagccatgaccaccgagacagcaatcatgcctggcagcagactgacccctagccagacaacctccgccggaaccaccggcaccggctctcataagagcagccgcgccccttctctggccgctacaatgaccctggagcctacagcttctaccagcctgagaatcaccgaaatctcccctcacagcagcaagatgaccaaggtggccattagcacatctgtgctgctggtgggcgccggcgtggtgatggccttcctggcttggtacatcaagagctga

SEQ ID NO: 12 - RNA, 1329 nt, synthetic construct
  source 1..1329: mol_type = other RNA
atgtatagcatgcagctggccagctgtgtgaccctgaccctggtgctgctggtgaactctgcccctacaagcagcagcacctccagcagcaccgctgaagcccagcagcagcagcagcagcaacaacagcagcaacagcacctggaacagctgctgatggacctgcaggagctgctgagccggatggaaaactacaggaacctgaagctgcccagaatgctgacctttaagttctacctgcctaagcaggccaccgagttgaaggacctgcaatgtctggaagatgaactgggccctctgagacacgtgctggacctgacacagagcaagtccttccagctggaagatgccgagaacttcatcagcaatatcagagtgaccgtggtgaagctgaaaggcagcgacaacaccttcgagtgccagttcgacgacgagagcgctacagttgtggacttcctgcggagatggatcgccttctgccaaagcattatcagcacctctcctcagagcggaggcggcagcggcggcggaggaagcggcggcggcggaagcggcggaggcggctccggcggcggatctctgcaggagctttgtctgtacgaccctccagaggtgcctaacgccacatttaaggccctgagctacaagaacggcaccatcctgaattgcgagtgcaagcggggctttagaagactgaaggaactggtctacatgcggtgcctgggtaacagctggtccagcaactgccagtgcaccagtaatagccacgacaagagcagaaagcaggtcacagctcagctggaacatcagaaagagcaacagaccaccacagacatgcagaagcctacccaaagcatgcaccaggagaacctgaccggccactgtagagagcctcctccatggaagcacgaggatagcaagagaatctaccacttcgtggaaggccagtctgtgcactacgagtgtatccccggctacaaagccctgcagagaggccccgccatcagcatctgcaagatgaaatgcggcaagaccggatggacccagccccagctgacatgcgtggatgagagagaacaccacagattcctcgcctctgaggagagccagggctctcggaactccagccctgagtctgagacatcctgccccatcacaacaacagatttccctcagcctaccgagactaccgccatgaccgaaaccttcgtgctgaccatggaatacaaggtggccgtggctagctgcctcttcctgctcatctctatcctgctgctgtccggcctgacctggcagcatagatggcggaagtctaggcgcaccatctga

SEQ ID NO: 13 - RNA, 576 nt, synthetic construct
  source 1..576: mol_type = other RNA
atgagagtgaccgcccccagaaccctgatcctgctgctgtctggcgccctggccctgacagagacatgggccggaagcggatcctgtgacctgcctcacacttataacctcgggaacaagagggccttgacagtcctggaagaaatgagaagactcccccctctttcctgcctgaaggacaggaaggattttggattccccttggagaaggtggataaccaacagatccagaaggctcaagccatccttgtgctaagagatcttacccagcagattttgaacctcttcacatcaaaagacttgtctgctacttggaatgcaactctcctagactcattctgcaatgacctccatcagcagctcaatgatctcaaagcctgtgtgatgcaggaacctcctctgacccaggaagactccctgctggctgtgaggacatacttccacaggatcactgtgtacctgagaaagaagaaacacagcctctgtgcctgggaggtgatcagagcagaagtctggagagccctctcttcctcaaccaacttgctggcaagactgagtgaggagaaggagtgataa

SEQ ID NO: 14 - RNA, 1638 nt, synthetic construct
  source 1..1638: mol_type = other RNA
atgagagtgaccgcccccagaaccctgatcctgctgctgtctggcgccctggccctgacagagacatgggccggaagcggatccatgtgggagctggagaaagacgtttatgttgtagaggtggactggactcccgatgcccctggagaaacagtgaacctcacctgtgacacgcctgaagaagatgacatcacctggacctcagaccagagacatggagtcataggctctggaaagaccctgaccatcactgtcaaagagtttctagatgctggccagtacacctgccacaaaggaggcgagactctgagccactcacatctgctgctccacaagaaggaaaatggaatttggtccactgaaattttaaaaaatttcaaaaacaagactttcctgaagtgtgaagcaccaaattactccggacggttcacgtgctcatggctggtgcaaagaaacatggacttgaagttcaacatcaagagcagtagcagttcccctgactctcgggcagtgacatgtggaatggcgtctctgtctgcagagaaggtcacactggaccaaagggactatgagaagtattcagtgtcctgccaggaggatgtcacctgcccaactgccgaggagaccctgcccattgaactggcgttggaagcacggcagcagaataaatatgagaactacagcaccagcttcttcatcagggacatcatcaaaccagacccgcccaagaacttgcagatgaagcctttgaagaactcacaggtggaggtcagctgggagtaccctgactcctggagcactccccattcctacttctccctcaagttctttgttcgaatccagcgcaagaaagaaaagatgaaggagacagaggaggggtgtaaccagaaaggtgcgttcctcgtagagaagacatctaccgaagtccaatgcaaaggcgggaatgtctgcgtgcaagctcaggatcgctattacaattcctcatgcagcaagtgggcatgtgttccctgcagagtccgatcggttcctggagtaggggtacctggagtgggcagggtcataccggtctctggacctgccaggtgtcttagccagtcccgaaacctgctgaagaccacagatgacatggtgaagacggccagagaaaagctgaaacattattcctgcactgctgaagacatcgatcatgaagacatcacacgggaccaaaccagcacattgaagacctgtttaccactggaactacacaagaacgagagttgcctggctactagagagacttcttccacaacaagagggagctgcctgcccccacagaagacgtctttgatgatgaccctgtgccttggtagcatctatgaggacttgaagatgtaccagacagagttccaggccatcaacgcagcacttcagaatcacaaccatcagcagatcattctagacaagggcatgctggtggccatcgatgagctgatgcagtctctgaatcataatggcgagactctgcgccagaaacctcctgtgggagaagcagacccttacagagtgaaaatgaagctctgcatcctgcttcacgccttcagcacccgcgtcgtgaccatcaacagggtgatgggctatctgtccagcgcctgataa

SEQ ID NO: 15 - RNA, 474 nt, synthetic construct
  source 1..474: mol_type = other RNA
atgggcgccatggctccaagaacactgctgctgctgctggctgccgctctggcccctacccagacaagagccggccctggaagcgagtgtcacatcaaggacaaggagggaaaggcttacgagagcgtgctgatgatcagcatcgatgagctggacaagatgacaggcaccgactctaactgccctaacaacgagcctaacttctttcgcaagcacgtgtgcgatgacaccaaggaggctgccttcctgaacagagccgctaggaagctgaagcagttcctgaagatgaacatcagcgaggagttcaacgtgcacctgctgaccgtgtctcagggaacccagacactggtgaactgtaccagcaaggaggagaagaacgtgaaggagcagaagaagaacgacgcctgctttctgaagaggctgctgagagagatcaagacctgctggaacaagatcctgaagggatccatctga

SEQ ID NO: 16 - RNA, 16 nt, synthetic construct
  source 1..16: mol_type = other RNA
ggctagcgccgccacc

SEQ ID NO: 17 - RNA, 839 nt, synthetic construct
  source 1..839: mol_type = other RNA
attctaactgcaacctttcgaagcctttgctctggcacaacaggtagtaggcgacactgttcgtgttgtcaacatgaccaacaagtgtctcctccaaattgctctcctgttgtgcttctccactacagctctttccatgagctacaacttgcttggattcctacaaagaagcagcaattttcagtgtcagaagctcctgtggcaattgaatgggaggcttgaatactgcctcaaggacaggatgaactttgacatccctgaggagattaagcagctgcagcagttccagaaggaggacgccgcattgaccatctatgagatgctccagaacatctttgctattttcagacaagattcatctagcactggctggaatgagactattgttgagaacctcctggctaatgtctatcatcagataaaccatctgaagacagtcctggaagaaaaactggagaaagaagatttcaccaggggaaaactcatgagcagtctgcacctgaaaagatattatgggaggattctgcattacctgaaggccaaggagtacagtcactgtgcctggaccatagtcagagtggaaatcctaaggaacttttacttcattaacagacttacaggttacctccgaaactgaagatctcctagcctgtgcctctgggactggacaattgcttcaagcattcttcaaccagcagatgctgtttaagtgactgatggctaatgtactgcatatgaaaggacactagaagattttgaaatttttattaaattatgagttatttttatttatttaaattttattttggaaaataaattatttttggtgcaaaagtcaa

SEQ ID NO: 18 - RNA, 1144 nt, synthetic construct
  source 1..1144: mol_type = other RNA
agaaagatcagttaagtcctttggacctgatcagcttgatacaagaactactgatttcaacttctttggcttaattctctcggaaacgatgaaatatacaagttatatcttggcttttcagctctgcatcgttttgggttctcttggctgttactgccaggacccatatgtaaaagaagcagaaaaccttaagaaatattttaatgcaggtcattcagatgtagcggataatggaactcttttcttaggcattttgaagaattggaaagaggagagtgacagaaaaataatgcagagccaaattgtctccttttacttcaaactttttaaaaactttaaagatgaccagagcatccaaaagagtgtggagaccatcaaggaagacatgaatgtcaagtttttcaatagcaacaaaaagaaacgagatgacttcgaaaagctgactaattattcggtaactgacttgaatgtccaacgcaaagcaatacatgaactcatccaagtgatggctgaactgtcgccagcagctaaaacagggaagcgaaaaaggagtcagatgctgtttcgaggtcgaagagcatcccagtaatggttgtcctgcctgcaatatttgaattttaaatctaaatctatttattaatatttaacattatttatatggggaatatatttttagactcatcaatcaaataagtatttataatagcaacttttgtgtaatgaaaatgaatatctattaatatatgtattatttataattcctatatcctgtgactgtctcacttaatcctttgttttctgactaattaggcaaggctatgtgattacaaggctttatctcaggggccaactaggcagccaacctaagcaagatcccatgggttgtgtgtttatttcacttgatgatacaatgaacacttataagtgaagtgatactatccagttactgccggtttgaaaatatgcctgcaatctgagccagtgctttaatggcatgtcagacagaacttgaatgtgtcaggtgaccctgatgaaaacatagcatctcaggagatttcatgcctggtgcttccaaatattgttgacaactgtgactgtacccaaatggaaagtaactcatttgttaaaattggggggggggggg

SEQ ID NO: 19 - RNA, 1620 nt, synthetic construct
  source 1..1620: mol_type = other RNA
atgtgtcatcagcagctggtcattagttggtttagcctggtcttcctggcatcacctctggtcgcaatctgggaactgaaaaaggacgtgtacgtggtggagctggactggtatccagatgcccctggcgagatggtggtgctgacctgtgataccccagaggaggacggcatcacatggaccctggaccagagctccgaggtgctgggcagcggcaagaccctgacaatccaggtgaaggagttcggcgatgccggccagtacacctgtcacaagggcggcgaggtgctgagccactccctgctgctgctgcacaagaaggaggatggcatctggtccaccgacatcctgaaggatcagaaggagcccaagaacaagaccttcctgagatgtgaggccaagaattacagcggcaggtttacctgctggtggctgacaaccatctccaccgatctgacattctccgtgaagagctccaggggcagctccgatccacagggcgtgacatgtggcgccgccacactgagcgccgagagagtgaggggcgacaacaaggagtacgagtactccgtggagtgtcaggaggactctgcctgtccagccgccgaggagtctctgccaatcgaggtaatggtggatgccgtgcacaagctgaagtacgagaactatacatccagctttttcatcagggacatcatcaagcccgatccacctaagaatctgcagctgaagccactgaagaactccagacaggtggaggtgtcttgggagtatccagatacctggtccacaccacactcttacttcagcctgaccttctgcgtgcaggtgcagggcaagtctaagcgggagaagaaggatcgcgtgtttaccgacaagacatccgccaccgtgatctgcaggaagaatgccagcatctccgtgagagcccaggatcggtattactcctctagctggagcgagtgggccagcgtgccatgcagcggctcttccggcggcggcggcagcccaggcggcggctcttcccggaatctgccagtggccacaccagatcccggcatgttcccctgtctgcaccacagccagaatctgctgagagccgtgtctaatatgctgcagaaggccagacagaccctggagttctacccctgcacctctgaggagatcgatcacgaggacatcaccaaggacaagacctccacagtggaggcctgcctgccactggagctgaccaagaacgagtcctgtctgaacagcagagagacctccttcatcacaaatggctcttgtctggcctccaggaagacatccttcatgatggccctgtgcctgagctctatctacgaggacctgaagatgtaccaggtggagttcaagacaatgaacgccaagctgctgatggatcccaagcgccagatcttcctggatcagaacatgctggccgtgatcgatgagctgatgcaggccctgaacttcaacagcgagacagtgccccagaagtcctctctggaggagccagatttctacaagaccaagatcaagctgtgcatcctgctgcacgcatttcgcattcgcgcagtgaccattgacagagtgatgagctacctgaacgccagctga

SEQ ID NO: 20 - RNA, 1620 nt, synthetic construct
  source 1..1620: mol_type = other RNA
atgtgccaccagcagctggtgatctcttggttttctctggtgttcctggccagccctctggtcgctatctgggagctgaaaaaagatgtgtacgtggtggaactggactggtaccctgatgcccctggagaaatggtcgtgctgacctgcgacacacctgaggaagatggaatcacatggacactggaccagagctctgaagtgctgggcagcgggaagaccctgacaatccaggtgaaagaatttggcgatgccggccagtacacctgtcacaagggcggcgaggtgctgtctcacagcttgctgctcctccacaaaaaggaagacggcatctggtccacagacatcctgaaggatcagaaggaacctaagaacaagaccttcctgcggtgcgaggccaaaaattacagcggaagattcacatgctggtggctgaccaccatcagcaccgacctgaccttcagcgtgaagtcctctaggggcagctctgatccacaaggcgtgacatgtggcgccgctacactgagcgctgagagagtgcggggcgacaacaaggagtacgagtactctgtcgagtgccaggaggacagcgcctgccccgccgctgaggaaagcctgcctatcgaggtgatggtggacgcagtgcacaagctgaaatacgagaactacacaagctccttcttcatcagagacatcatcaagcctgatcctcctaagaacctgcaactgaagcccctgaagaatagcagacaggtggaagtcagctgggagtatcccgatacatggtccacaccccacagttatttcagcctgaccttttgcgtgcaggtgcagggcaagagcaagcgggaaaagaaggaccgggtgttcaccgacaagacctccgccaccgtgatctgcagaaagaacgcctctatcagcgtgcgggctcaggacagatactacagcagtagctggtcagagtgggccagcgtgccatgcagcggcagcagcggcggaggcggatctccaggcggcggcagcagccggaacctgcctgtggccacccccgaccctggcatgttcccatgtctccatcacagccagaacctgctgagagccgtgtccaacatgctgcagaaggccagacaaacactggagttctacccctgtacaagcgaggaaatcgaccacgaggacattaccaaggacaagacctctaccgtggaagcttgtcttcctcttgagctgaccaagaatgagagctgcctgaacagcagagagacttcctttatcaccaacggctcttgcctggccagccgcaagacgagctttatgatggccctgtgtctgagcagcatctacgaggacctgaaaatgtaccaggttgagttcaagaccatgaacgccaagctgctgatggaccctaagagacagatcttcctggaccagaacatgctggctgtgattgatgagctgatgcaggccctgaacttcaacagcgaaaccgtgcctcagaaaagcagcctggaagagcccgacttctacaagaccaagatcaagctgtgcatcctgctgcacgccttcagaatccgggccgtgaccatcgatagagtgatgagctacctgaatgcctcctga

SEQ ID NO: 21 - RNA, 1620 nt, synthetic construct
  source 1..1620: mol_type = other RNA
atgtgccaccagcagctggtgatcagctggttcagccttgtgttcctggccagccctctggtggccatctgggagctgaaaaaagacgtgtacgtggtggaactggactggtacccagatgcccctggcgagatggtggtgctgacctgcgacacccctgaggaagacggcatcacctggaccctggatcagagcagcgaggtgctcggctctggcaagaccctgaccatccaagtgaaggagttcggcgatgccggccagtacacctgtcacaagggcggagaagtgctgagccacagcctgctgctgctgcataagaaggaggatggcatctggtctacagacattctgaaggaccagaaagaacctaagaacaaaaccttcctgcggtgcgaggccaagaattactctggccggttcacctgttggtggctcacaaccatcagcacagacctgacatttagcgtgaagtcatccagaggcagcagcgacccacagggcgtgacctgcggtgctgccaccctttctgccgagagggtgcggggcgacaacaaggagtatgagtacagcgtggaatgccaggaggacagcgcctgccctgccgctgaagagagcctgcccatcgaggtgatggtcgacgccgtgcacaagctgaagtacgagaactacaccagcagctttttcatccgggacatcatcaagcctgatccacctaagaacctgcagctgaagcccctgaaaaacagccgccaggtcgaagtgtcctgggaatatcctgacacatggagcacccctcacagctacttcagcctgaccttctgcgtccaggtccagggaaagtccaagagagaaaagaaagacagagttttcaccgataagacaagcgccacagtgatctgcagaaaaaatgctagcatctcagtgcgggcccaggacagatactacagctccagttggagcgagtgggccagcgtgccctgcagcggaagctctggcggaggcggcagccccggcggcggctcctcacggaacctgcccgtggccacacctgatcccggcatgttcccctgtctgcaccactctcagaacctgctcagagctgtgtctaatatgctgcaaaaggccagacagaccctcgagttctacccctgcacctccgaggaaatcgaccacgaggacatcacaaaggacaagacaagcaccgtggaagcctgtctgcctctggagctgacaaagaacgagagctgcctgaatagcagagagacatcttttatcacaaacggcagttgtctggccagccggaagaccagcttcatgatggccctgtgcctgtctagcatctacgaggatctgaagatgtaccaggtggagttcaagaccatgaacgccaagctgctgatggaccctaaaagacaaatcttcctggaccaaaacatgctggctgttattgatgagctgatgcaggccctgaacttcaactctgaaaccgtgcctcagaaatccagcctggaagagcctgacttctataagaccaagatcaagctgtgcatcctgctgcacgcctttagaatcagagccgtgaccatcgatagagtgatgagctacctgaacgcttcttga

SEQ ID NO: 22 - RNA, 534 nt, synthetic construct
  source 1..534: mol_type = other RNA
atgtttcacgtgtctttccggtacatcttcggcctgccacctctgatcctggtgctgctgccagtggcctccagcgattgcgacatcgagggcaaggatggcaagcagtacgagagcgtgctgatggtgtccatcgatcagctgctggacagcatgaaggagatcggcagcaactgcctgaataacgagttcaactttttcaagaggcacatctgtgacgccaataaggagggcatgtttctgttcagagccgccagaaagctgaggcagttcctgaagatgaacagcaccggcgatttcgacctgcacctgctgaaggtgtctgagggcacaaccatcctgctgaattgcaccggccaggtgaagggcaggaagccagccgccctgggcgaggcccagcctacaaagagcctggaggagaacaagagcctgaaggagcagaagaagctgaatgacctgtgcttcctgaagagactgctgcaggagatcaagacctgttggaacaagatcctgatgggcaccaaggagcactga

SEQ ID NO: 23 - RNA, 534 nt, synthetic construct
  source 1..534: mol_type = other RNA
atgtttcacgtgtccttccgctacatcttcggcctgccacctctgatcctggtgctgctgcctgtggccagcagcgactgcgacatcgagggcaaggacggcaaacagtacgagagcgtgctgatggtcagcatcgaccagctgctggatagcatgaaggaaatcggctctaattgtctgaacaacgagttcaacttcttcaagcggcacatctgcgatgccaacaaagaaggcatgttcctgttccgggccgccagaaagctgagacaatttctgaagatgaacagcaccggagatttcgacctgcatctgctgaaggtgtccgagggaaccacaatcctgctgaattgcaccggccaggtgaagggcagaaagcccgctgctctgggcgaggcccagcctacaaagagccttgaggaaaacaagtctctgaaggaacagaaaaagctgaacgacctgtgcttcctgaaaagactgctccaggagattaagacctgttggaacaagatcctgatgggcaccaaggaacactga

SEQ ID NO: 24 - RNA, 534 nt, synthetic construct
  source 1..534: mol_type = other RNA
atgttccatgtgtccttccggtacatcttcggcctgcctccactgatcctggtgctgctccccgtggcctctagcgactgcgatatcgagggcaaggacggcaaacagtacgagagcgtgctgatggtcagcatcgaccagctgctggacagcatgaaggaaatcggcagcaactgcctgaacaacgagttcaacttcttcaagcgccacatctgtgatgccaacaaggaaggaatgttcctctttagagccgctagaaagctgagacaatttctgaagatgaactctacaggagatttcgacctgcacctgctgaaggtgtccgagggcaccaccatcctgctgaattgcaccggccaggtgaagggcagaaagcctgctgccctgggcgaggcccagcctaccaagagcctggaagagaacaaaagcctgaaagaacagaaaaagctgaatgacctgtgcttcctgaagcggctgctgcaggagattaagacctgttggaacaagatcctgatgggcacaaaggaacactga

SEQ ID NO: 25 - RNA, 426 nt, synthetic construct
  source 1..426: mol_type = other RNA
atgtggctgcagaacctgctgtttctgggaatcgtggtgtacagtctgtccgcccccaccagaagcccaatcactgtgaccagaccctggaagcacgtggaggccatcaaagaggctctgaatctgctggatgacatgcccgtgactctgaatgaggaagtggaggtggtgagcaacgagttcagctttaagaagctgacctgcgtgcagacaaggctgaagatctttgagcagggcctgaggggaaactttactaagctgaagggtgccctgaatatgacagcctcttactatcagacctactgcccacccactcctgagactgattgtgagacccaggtgacaacatacgccgacttcatcgacagcctgaagaccttcctgaccgatatccccttcgagtgcaagaagcccggccagaagtga

SEQ ID NO: 26 - RNA, 567 nt, synthetic construct
  source 1..567: mol_type = other RNA
atggccctgacatttgccctgctggtggccctgctggtgctgagctgcaagtcttcctgcagcgtgggctgtgatctgccacagacccactccctgggcagcagaaggaccctgatgctgctggcccagatgcggagaatcagcctgttctcttgcctgaaggatagacacgactttggcttcccacaggaggagtttggcaaccagttccagaaggccgagacaatcccagtgctgcacgagatgatccagcagatcttcaacctgttcagcacaaaggacagctctgccgcctgggatgagacactgctggataagttctacaccgagctgtatcagcagctgaatgacctggaggcctgcgtgatccagggcgtgggcgtgaccgagacaccactgatgaaggaggatagcatcctggccgtgaggaagtacttccagagaatcaccctgtatctgaaggagaagaagtacagcccctgtgcctgggaggtggtgcgggccgagatcatgcggtcctttagcctgtccaccaatctgcaggagtctctgagaagcaaggagtga

SEQ ID NO: 27 - RNA, 567 nt, synthetic construct
  source 1..567: mol_type = other RNA
atggccctcaccttcgccctgctggtcgccctgctggtgctgagctgcaagtcctcctgcagcgtgggatgtgatctgcctcagacccacagcctgggcagcagaaggaccctgatgctgctggcccagatgcggagaatcagcctgttttcttgtctgaaagatagacacgacttcggctttccacaggaggagttcggcaaccagttccagaaggccgagacaattcctgtgctgcacgagatgatccaacagatcttcaacctgttcagcaccaaggactcttctgccgcttgggacgagacactgcttgataagttctacaccgagctgtatcagcagctgaacgacctggaagcctgcgtgatccagggcgtgggcgtgaccgagacacctctgatgaaagaggacagcatcctggctgttcggaagtacttccaaagaatcaccctgtacctgaaggaaaagaagtacagcccctgcgcctgggaggtggtgcgggccgaaatcatgagaagcttcagcctgtctacaaatctgcaggagagcctgagaagcaaggaatga

SEQ ID NO: 28 - RNA, 567 nt, synthetic construct
  source 1..567: mol_type = other RNA
atggccctgaccttcgccctgctggtggccctgctggttctgtcttgtaaaagcagctgcagcgtgggctgcgacctgccacagacacactctctgggaagcagaagaaccctgatgctgctggcccagatgcggcggatcagcctctttagctgcctgaaagatagacacgacttcggcttccctcaggaggagttcggcaaccagttccagaaggccgagacaatccccgtgctgcacgagatgatccagcaaatctttaatctgttcagcaccaaggacagctccgccgcttgggatgagacactcctggacaagttctacaccgagctgtaccagcagctgaacgacctggaagcttgtgtgattcagggcgtgggcgtgaccgagacccctctgatgaaggaagatagcatcctggccgtgcggaagtacttccaaagaatcacactgtacctgaaggagaagaagtatagcccttgcgcctgggaggtggtcagagccgaaatcatgagaagcttctccctgagcaccaacctgcaggagtctctgagatccaaggaatga

SEQ ID NO: 29 - RNA, 728 nt, synthetic construct
  source 1..728: mol_type = other RNA
atggccccgcggcgggcgcgcggctgccggaccctcggtctcccggcgctgctactgctgctgctgctccggccgccggcgacgcggggcatcacgtgccctccccccatgtccgtggaacacgcagacatctgggtcaagagctacagcttgtactccagggagcggtacatttgtaactctggtttcaagcgtaaagccggcacgtccagcctgacggagtgcgtgttgaacaaggccacgaatgtcgcccactggacaacccccagtctcaaatgcattagagaccctgccctggttcaccaaaggccagcgccacccgggggaggatctggcggcggtgggtctggcgggggatctggcggaggaggaagcttacagaactgggtgaatgtaataagtgatttgaaaaaaattgaagatcttattcaattctatgcatattgatgctactttatatacggaaagtgatgttcaccccagttgcaaagtaacagcaatgaagtgctttctcttggagttacaagttatttcacttgagtccggagatgcaagtattcatgatacagtagaaaattatcatcctagcaaacaacagtttgtcttctaatgggaatgtaacagaatctggatgcaaagaatgtgaggaactggaggaaaaaaatattaaagaatttttgcagagttttgtacatattgtccaaatgttcatcaacacttcttgatga

SEQ ID NO: 30 - DNA, 12 bp, synthetic construct
  source 1..12: mol_type = other DNA
cgtcaacgtcgt

SEQ ID NO: 31 - RNA, 12 nt, synthetic construct
  source 1..12: mol_type = other RNA
cgtcaacgtcgt

SEQ ID NO: 32 - protein, 25 aa, synthetic construct
GSGVKQTLNFDLLKLAGDVESNPGP

SEQ ID NO: 33 - protein, 22 aa, synthetic construct
GSGATNFSLLKQAGDVEENPGP

SEQ ID NO: 34 - protein, 21 aa, synthetic construct
GSGEGRGSLLTCGDVEENPGP

SEQ ID NO: 35 - protein, 23 aa, synthetic construct
GSGQCTNYALLKLAGDVESNPGP

SEQ ID NO: 36 - RNA, 66 nt, synthetic construct
  source 1..66: mol_type = other RNA
ggaagcggagctactaacttcagcctgctgaagcaggctggagacgtggaggagaaccctggacct

SEQ ID NO: 37 - RNA, 108 nt, synthetic construct
  source 1..108: mol_type = other RNA
tccggactcagatccggggatctcaaaattgtcgctcctgtcaaacaaactcttaactttgatttactcaaactggctggggatgtagaaagcaatccaggtccactc

SEQ ID NO: 38 - RNA, 34 nt, synthetic construct
  source 1..34: mol_type = other RNA
gagacccaagctggctagcgggagaaagcttacc

SEQ ID NO: 39 - protein, 197 aa, synthetic construct
RNLPVATPDPGMFPCLHHSQNLLRAVSNMLQKARQTLEFYPCTSEEIDHEDITKDKTSTVEACLPLELTKNESCLNSRETSFITNGSCLASRKTSFMMALCLSSIYEDLKMYQVEFKTMNAKLLMDPKRQIFLDQNMLAVIDELMQALNFNSETVPQKSSLEEPDFYKTKIKLCILLHAFRIRAVTIDRVMSYLNAS

SEQ ID NO: 40 - protein, 328 aa, synthetic construct
MCHQQLVISWFSLVFLASPLVAIWELKKDVYVVELDWYPDAPGEMVVLTCDTPEEDGITWTLDQSSEVLGSGKTLTIQVKEFGDAGQYTCHKGGEVLSHSLLLLHKKEDGIWSTDILKDQKEPKNKTFLRCEAKNYSGRFTCWWLTTISTDLTFSVKSSRGSSDPQGVTCGAATLSAERVRGDNKEYEYSVECQEDSACPAAEESLPIEVMVDAVHKLKYENYTSSFFIRDIIKPDPPKNLQLKPLKNSRQVEVSWEYPDTWSTPHSYFSLTFCVQVQGKSKREKKDRVFTDKTSATVICRKNASISVRAQDRYYSSSWSEWASVPCS

SEQ ID NO: 41 - protein, 14 aa, synthetic construct
GSSGGGGSPGGGSS

SEQ ID NO: 42 - protein, 177 aa, synthetic construct
MFHVSFRYIFGLPPLILVLLPVASSDCDIEGKDGKQYESVLMVSIDQLLDSMKEIGSNCLNNEFNFFKRHICDANKEGMFLFRAARKLRQFLKMNSTGDFDLHLLKVSEGTTILLNCTGQVKGRKPAALGEAQPTKSLEENKSLKEQKKLNDLCFLKRLLQEIKTCWNKILMGTKEH

SEQ ID NO: 43 - protein, 188 aa, synthetic construct
MALTFALLVALLVLSCKSSCSVGCDLPQTHSLGSRRTLMLLAQMRRISLFSCLKDRHDFGFPQEEFGNQFQKAETIPVLHEMIQQIFNLFSTKDSSAAWDETLLDKFYTELYQQLNDLEACVIQGVGVTETPLMKEDSILAVRKYFQRITLYLKEKKYSPCAWEVVRAEIMRSFSLSTNLQESLRSKE

SEQ ID NO: 44 - DNA, 1620 bp, synthetic construct
  source 1..1620: mol_type = other DNA
atgtgtcatcagcagctggtcattagttggtttagcctggtcttcctggcatcacctctggtcgcaatctgggaactgaaaaaggacgtgtacgtggtggagctggactggtatccagatgcccctggcgagatggtggtgctgacctgtgataccccagaggaggacggcatcacatggaccctggaccagagctccgaggtgctgggcagcggcaagaccctgacaatccaggtgaaggagttcggcgatgccggccagtacacctgtcacaagggcggcgaggtgctgagccactccctgctgctgctgcacaagaaggaggatggcatctggtccaccgacatcctgaaggatcagaaggagcccaagaacaagaccttcctgagatgtgaggccaagaattacagcggcaggtttacctgctggtggctgacaaccatctccaccgatctgacattctccgtgaagagctccaggggcagctccgatccacagggcgtgacatgtggcgccgccacactgagcgccgagagagtgaggggcgacaacaaggagtacgagtactccgtggagtgtcaggaggactctgcctgtccagccgccgaggagtctctgccaatcgaggtaatggtggatgccgtgcacaagctgaagtacgagaactatacatccagctttttcatcagggacatcatcaagcccgatccacctaagaatctgcagctgaagccactgaagaactccagacaggtggaggtgtcttgggagtatccagatacctggtccacaccacactcttacttcagcctgaccttctgcgtgcaggtgcagggcaagtctaagcgggagaagaaggatcgcgtgtttaccgacaagacatccgccaccgtgatctgcaggaagaatgccagcatctccgtgagagcccaggatcggtattactcctctagctggagcgagtgggccagcgtgccatgcagcggctcttccggcggcggcggcagcccaggcggcggctcttcccggaatctgccagtggccacaccagatcccggcatgttcccctgtctgcaccacagccagaatctgctgagagccgtgtctaatatgctgcagaaggccagacagaccctggagttctacccctgcacctctgaggagatcgatcacgaggacatcaccaaggacaagacctccacagtggaggcctgcctgccactggagctgaccaagaacgagtcctgtctgaacagcagagagacctccttcatcacaaatggctcttgtctggcctccaggaagacatccttcatgatggccctgtgcctgagctctatctacgaggacctgaagatgtaccaggtggagttcaagacaatgaacgccaagctgctgatggatcccaagcgccagatcttcctggatcagaacatgctggccgtgatcgatgagctgatgcaggccctgaacttcaacagcgagacagtgccccagaagtcctctctggaggagccagatttctacaagaccaagatcaagctgtgcatcctgctgcacgcatttcgcattcgcgcagtgaccattgacagagtgatgagctacctgaacgccagctga

SEQ ID NO: 45 - DNA, 1620 bp, synthetic construct
  source 1..1620: mol_type = other DNA
atgtgccaccagcagctggtgatctcttggttttctctggtgttcctggccagccctctggtcgctatctgggagctgaaaaaagatgtgtacgtggtggaactggactggtaccctgatgcccctggagaaatggtcgtgctgacctgcgacacacctgaggaagatggaatcacatggacactggaccagagctctgaagtgctgggcagcgggaagaccctgacaatccaggtgaaagaatttggcgatgccggccagtacacctgtcacaagggcggcgaggtgctgtctcacagcttgctgctcctccacaaaaaggaagacggcatctggtccacagacatcctgaaggatcagaaggaacctaagaacaagaccttcctgcggtgcgaggccaaaaattacagcggaagattcacatgctggtggctgaccaccatcagcaccgacctgaccttcagcgtgaagtcctctaggggcagctctgatccacaaggcgtgacatgtggcgccgctacactgagcgctgagagagtgcggggcgacaacaaggagtacgagtactctgtcgagtgccaggaggacagcgcctgccccgccgctgaggaaagcctgcctatcgaggtgatggtggacgcagtgcacaagctgaaatacgagaactacacaagctccttcttcatcagagacatcatcaagcctgatcctcctaagaacctgcaactgaagcccctgaagaatagcagacaggtggaagtcagctgggagtatcccgatacatggtccacaccccacagttatttcagcctgaccttttgcgtgcaggtgcagggcaagagcaagcgggaaaagaaggaccgggtgttcaccgacaagacctccgccaccgtgatctgcagaaagaacgcctctatcagcgtgcgggctcaggacagatactacagcagtagctggtcagagtgggccagcgtgccatgcagcggcagcagcggcggaggcggatctccaggcggcggcagcagccggaacctgcctgtggccacccccgaccctggcatgttcccatgtctccatcacagccagaacctgctgagagccgtgtccaacatgctgcagaaggccagacaaacactggagttctacccctgtacaagcgaggaaatcgaccacgaggacattaccaaggacaagacctctaccgtggaagcttgtcttcctcttgagctgaccaagaatgagagctgcctgaacagcagagagacttcctttatcaccaacggctcttgcctggccagccgcaagacgagctttatgatggccctgtgtctgagcagcatctacgaggacctgaaaatgtaccaggttgagttcaagaccatgaacgccaagctgctgatggaccctaagagacagatcttcctggaccagaacatgctggctgtgattgatgagctgatgcaggccctgaacttcaacagcgaaaccgtgcctcagaaaagcagcctggaagagcccgacttctacaagaccaagatcaagctgtgcatcctgctgcacgccttcagaatccgggccgtgaccatcgatagagtgatgagctacctgaatgcctcctga

SEQ ID NO: 46 - DNA, 1620 bp, synthetic construct
  source 1..1620: mol_type = other DNA
atgtgccaccagcagctggtgatcagctggttcagccttgtgttcctggccagccctctggtggccatctgggagctgaaaaaagacgtgtacgtggtggaactggactggtacccagatgcccctggcgagatggtggtgctgacctgcgacacccctgaggaagacggcatcacctggaccctggatcagagcagcgaggtgctcggctctggcaagaccctgaccatccaagtgaaggagttcggcgatgccggccagtacacctgtcacaagggcggagaagtgctgagccacagcctgctgctgctgcataagaaggaggatggcatctggtctacagacattctgaaggaccagaaagaacctaagaacaaaaccttcctgcggtgcgaggccaagaattactctggccggttcacctgttggtggctcacaaccatcagcacagacctgacatttagcgtgaagtcatccagaggcagcagcgacccacagggcgtgacctgcggtgctgccaccctttctgccgagagggtgcggggcgacaacaaggagtatgagtacagcgtggaatgccaggaggacagcgcctgccctgccgctgaagagagcctgcccatcgaggtgatggtcgacgccgtgcacaagctgaagtacgagaactacaccagcagctttttcatccgggacatcatcaagcctgatccacctaagaacctgcagctgaagcccctgaaaaacagccgccaggtcgaagtgtcctgggaatatcctgacacatggagcacccctcacagctacttcagcctgaccttctgcgtccaggtccagggaaagtccaagagagaaaagaaagacagagttttcaccgataagacaagcgccacagtgatctgcagaaaaaatgctagcatctcagtgcgggcccaggacagatactacagctccagttggagcgagtgggccagcgtgccctgcagcggaagctctggcggaggcggcagccccggcggcggctcctcacggaacctgcccgtggccacacctgatcccggcatgttcccctgtctgcaccactctcagaacctgctcagagctgtgtctaatatgctgcaaaaggccagacagaccctcgagttctacccctgcacctccgaggaaatcgaccacgaggacatcacaaaggacaagacaagcaccgtggaagcctgtctgcctctggagctgacaaagaacgagagctgcctgaatagcagagagacatcttttatcacaaacggcagttgtctggccagccggaagaccagcttcatgatggccctgtgcctgtctagcatctacgaggatctgaagatgtaccaggtggagttcaagaccatgaacgccaagctgctgatggaccctaaaagacaaatcttcctggaccaaaacatgctggctgttattgatgagctgatgcaggccctgaacttcaactctgaaaccgtgcctcagaaatccagcctggaagagcctgacttctataagaccaagatcaagctgtgcatcctgctgcacgcctttagaatcagagccgtgaccatcgatagagtgatgagctacctgaacgcttcttga

SEQ ID NO: 47 - DNA, 534 bp, synthetic construct
  source 1..534: mol_type = other DNA
atgtttcacgtgtctttccggtacatcttcggcctgccacctctgatcctggtgctgctgccagtggcctccagcgattgcgacatcgagggcaaggatggcaagcagtacgagagcgtgctgatggtgtccatcgatcagctgctggacagcatgaaggagatcggcagcaactgcctgaataacgagttcaactttttcaagaggcacatctgtgacgccaataaggagggcatgtttctgttcagagccgccagaaagctgaggcagttcctgaagatgaacagcaccggcgatttcgacctgcacctgctgaaggtgtctgagggcacaaccatcctgctgaattgcaccggccaggtgaagggcaggaagccagccgccctgggcgaggcccagcctacaaagagcctggaggagaacaagagcctgaaggagcagaagaagctgaatgacctgtgcttcctgaagagactgctgcaggagatcaagacctgttggaacaagatcctgatgggcaccaaggagcactga

SEQ ID NO: 48 - DNA, 534 bp, synthetic construct
  source 1..534: mol_type = other DNA
atgtttcacgtgtccttccgctacatcttcggcctgccacctctgatcctggtgctgctgcctgtggccagcagcgactgcgacatcgagggcaaggacggcaaacagtacgagagcgtgctgatggtcagcatcgaccagctgctggatagcatgaaggaaatcggctctaattgtctgaacaacgagttcaacttcttcaagcggcacatctgcgatgccaacaaagaaggcatgttcctgttccgggccgccagaaagctgagacaatttctgaagatgaacagcaccggagatttcgacctgcatctgctgaaggtgtccgagggaaccacaatcctgctgaattgcaccggccaggtgaagggcagaaagcccgctgctctgggcgaggcccagcctacaaagagccttgaggaaaacaagtctctgaaggaacagaaaaagctgaacgacctgtgcttcctgaaaagactgctccaggagattaagacctgttggaacaagatcctgatgggcaccaaggaacactga

SEQ ID NO: 49 - DNA, 534 bp, synthetic construct
  source 1..534: mol_type = other DNA
atgttccatgtgtccttccggtacatcttcggcctgcctccactgatcctggtgctgctccccgtggcctctagcgactgcgatatcgagggcaaggacggcaaacagtacgagagcgtgctgatggtcagcatcgaccagctgctggacagcatgaaggaaatcggcagcaactgcctgaacaacgagttcaacttcttcaagcgccacatctgtgatgccaacaaggaaggaatgttcctctttagagccgctagaaagctgagacaatttctgaagatgaactctacaggagatttcgacctgcacctgctgaaggtgtccgagggcaccaccatcctgctgaattgcaccggccaggtgaagggcagaaagcctgctgccctgggcgaggcccagcctaccaagagcctggaagagaacaaaagcctgaaagaacagaaaaagctgaatgacctgtgcttcctgaagcggctgctgcaggagattaagacctgttggaacaagatcctgatgggcacaaaggaacactga

SEQ ID NO: 50 - DNA, 567 bp, synthetic construct
  source 1..567: mol_type = other DNA
atggccctgacatttgccctgctggtggccctgctggtgctgagctgcaagtcttcctgcagcgtgggctgtgatctgccacagacccactccctgggcagcagaaggaccctgatgctgctggcccagatgcggagaatcagcctgttctcttgcctgaaggatagacacgactttggcttcccacaggaggagtttggcaaccagttccagaaggccgagacaatcccagtgctgcacgagatgatccagcagatcttcaacctgttcagcacaaaggacagctctgccgcctgggatgagacactgctggataagttctacaccgagctgtatcagcagctgaatgacctggaggcctgcgtgatccagggcgtgggcgtgaccgagacaccactgatgaaggaggatagcatcctggccgtgaggaagtacttccagagaatcaccctgtatctgaaggagaagaagtacagcccctgtgcctgggaggtggtgcgggccgagatcatgcggtcctttagcctgtccaccaatctgcaggagtctctgagaagcaaggagtga

SEQ ID NO: 51 - DNA, 567 bp, synthetic construct
  source 1..567: mol_type = other DNA
atggccctcaccttcgccctgctggtcgccctgctggtgctgagctgcaagtcctcctgcagcgtgggatgtgatctgcctcagacccacagcctgggcagcagaaggaccctgatgctgctggcccagatgcggagaatcagcctgttttcttgtctgaaagatagacacgacttcggctttccacaggaggagttcggcaaccagttccagaaggccgagacaattcctgtgctgcacgagatgatccaacagatcttcaacctgttcagcaccaaggactcttctgccgcttgggacgagacactgcttgataagttctacaccgagctgtatcagcagctgaacgacctggaagcctgcgtgatccagggcgtgggcgtgaccgagacacctctgatgaaagaggacagcatcctggctgttcggaagtacttccaaagaatcaccctgtacctgaaggaaaagaagtacagcccctgcgcctgggaggtggtgcgggccgaaatcatgagaagcttcagcctgtctacaaatctgcaggagagcctgagaagcaaggaatga

SEQ ID NO: 52 - DNA, 567 bp, synthetic construct
  source 1..567: mol_type = other DNA
atggccctgaccttcgccctgctggtggccctgctggttctgtcttgtaaaagcagctgcagcgtgggctgcgacctgccacagacacactctctgggaagcagaagaaccctgatgctgctggcccagatgcggcggatcagcctctttagctgcctgaaagatagacacgacttcggcttccctcaggaggagttcggcaaccagttccagaaggccgagacaatccccgtgctgcacgagatgatccagcaaatctttaatctgttcagcaccaaggacagctccgccgcttgggatgagacactcctggacaagttctacaccgagctgtaccagcagctgaacgacctggaagcttgtgtgattcagggcgtgggcgtgaccgagacccctctgatgaaggaagatagcatcctggccgtgcggaagtacttccaaagaatcacactgtacctgaaggagaagaagtatagcccttgcgcctgggaggtggtcagagccgaaatcatgagaagcttctccctgagcaccaacctgcaggagtctctgagatccaaggaatga